European Patent Application EP 4 710 930 A1, published March 18, 2026. Title: 잔탄검 또는 후코이단 포함하는 항인플루엔자 바이러스용 조성물. Applicant: 주식회사 대웅제약. Application KR. The sequence listing filed with the application follows.

SEQUENCE LISTING (6 sequences)

SEQ ID NO: 1 - DNA, 23 bp, synthetic construct
  source 1..23: mol_type = other DNA
cttctaaccgaggtcgaaacgta

SEQ ID NO: 2 - DNA, 25 bp, synthetic construct
  source 1..25: mol_type = other DNA
ggtgacaggattggtcttgtcttta

SEQ ID NO: 3 - DNA, 21 bp, synthetic construct
  source 1..21: mol_type = other DNA
tcaggccccctcaaagccgag

SEQ ID NO: 4 - DNA, 19 bp, synthetic construct
  source 1..19: mol_type = other DNA
cggtccaaattcctgctga

SEQ ID NO: 5 - DNA, 20 bp, synthetic construct
  source 1..20: mol_type = other DNA
cattgggttccttccatcca

SEQ ID NO: 6 - DNA, 29 bp, synthetic construct
  source 1..29: mol_type = other DNA
ccaagtcatgaaggagagggaataccgct